European Patent Specification EP 3 487 523 B1, published September 6, 2023. Title: THERAPEUTIC APPLICATIONS OF CPF1-BASED GENOME EDITING. Applicant: DUKE UNIVERSITY. The sequence listing filed with the application follows.

SEQUENCE LISTING (125 sequences)

SEQ ID NO: 1 - DNA, 27 bp, Homo sapiens
tttgcaaaaacccaaaatattttagct

SEQ ID NO: 2 - DNA, 27 bp, Homo sapiens
tttgcctttttggtatcttacaggaac

SEQ ID NO: 3 - DNA, 27 bp, Homo sapiens
tccaggatggcattgggcagcggcaaa

SEQ ID NO: 4 - DNA, 27 bp, Homo sapiens
tttatttttccttttattctagttgaa

SEQ ID NO: 5 - DNA, 27 bp, Homo sapiens
tttcttgatccatatgcttttacctgc

SEQ ID NO: 6 - DNA, 27 bp, Homo sapiens
aggcgatttgacagatctgttgagaaa

SEQ ID NO: 7 - DNA, 27 bp, Homo sapiens
tttattcttctttctccaggctagaag

SEQ ID NO: 8 - DNA, 27 bp, Homo sapiens
ttctttctccaggctagaagaacaaaa

SEQ ID NO: 9 - DNA, 27 bp, Homo sapiens
tacaggcaacaatgcaggatttggaac

SEQ ID NO: 10 - DNA, 27 bp, Homo sapiens
ttttctgttaaagaggaagttagaaga

SEQ ID NO: 11 - DNA, 27 bp, Homo sapiens
ttttaaaatttttatattacagaatat

SEQ ID NO: 12 - DNA, 27 bp, Homo sapiens
agaatataaaagatagtctacaacaaa

SEQ ID NO: 13 - DNA, 27 bp, Homo sapiens
tttattttgcattttagatgaaagaga

SEQ ID NO: 14 - DNA, 27 bp, Homo sapiens
ttttagatgaaagagaagatgttcaaa

SEQ ID NO: 15 - DNA, 27 bp, Homo sapiens
gatgaaagagaagatgttcaaaagaaa

SEQ ID NO: 16 - DNA, 27 bp, Homo sapiens
tttgcaaaaacccaaaatattttagct

SEQ ID NO: 17 - DNA, 27 bp, Homo sapiens
tttagcttgtgtttctaatttttcttt

SEQ ID NO: 18 - DNA, 27 bp, Homo sapiens
tttgacttattgttattgaaattggct

SEQ ID NO: 19 - DNA, 27 bp, Homo sapiens
tttctaccatgtattgctaaacaaagt

SEQ ID NO: 20 - DNA, 27 bp, Homo sapiens
tttagtatcaattcacaccagcaagtt

SEQ ID NO: 21 - DNA, 27 bp, Homo sapiens
ataatcgccactttacagaggagtaaa

SEQ ID NO: 22 - DNA, 27 bp, Homo sapiens
tttctttaaaatgaagattttccacca

SEQ ID NO: 23 - DNA, 27 bp, Homo sapiens
tttaaaatgaagattttccaccaatca

SEQ ID NO: 24 - DNA, 27 bp, Homo sapiens
ttttccaccaatcactttactctccta

SEQ ID NO: 25 - DNA, 27 bp, Homo sapiens
tttcccaccagttcttaggcaactgtt

SEQ ID NO: 26 - DNA, 27 bp, Homo sapiens
ataatcaaggatataaattaatgcaaa

SEQ ID NO: 27 - DNA, 27 bp, Homo sapiens
ttttgttgttgttgttaaggtcaaagt

SEQ ID NO: 28 - DNA, 27 bp, Homo sapiens
tttaaaattaccctagatcttaaagtt

SEQ ID NO: 29 - DNA, 28 bp, Homo sapiens
cacgcccccaccctaatcagaggccaaa

SEQ ID NO: 30 - DNA, 28 bp, Homo sapiens
ccaaacccttcctggagcctgtgataaa

SEQ ID NO: 31 - DNA, 28 bp, Homo sapiens
ccttccgaaagaggcccccctgggcaaa

SEQ ID NO: 32 - DNA, 28 bp, Homo sapiens
tctccatcaccaagagagccttccgaaa

SEQ ID NO: 33 - DNA, 28 bp, Homo sapiens
tgttagcttgcactagactagcttcaaa

SEQ ID NO: 34 - DNA, 28 bp, Homo sapiens
ttttctggcctatgttattacctgtatg

SEQ ID NO: 35 - DNA, 28 bp, Homo sapiens
tttctggcctatgttattacctgtatgg

SEQ ID NO: 36 - DNA, 23 bp, Artificial Sequence
  Synthetic
caaaaacccaaaatattttagct

SEQ ID NO: 37 - DNA, 23 bp, Artificial Sequence
  Synthetic
cctttttggtatcttacaggaac

SEQ ID NO: 38 - DNA, 23 bp, Artificial Sequence
  Synthetic
ccgctgcccaatgccatcctgga

SEQ ID NO: 39 - DNA, 23 bp, Artificial Sequence
  Synthetic
tttttccttttattctagttgaa

SEQ ID NO: 40 - DNA, 23 bp, Artificial Sequence
  Synthetic
ttgatccatatgcttttacctgc

SEQ ID NO: 41 - DNA, 23 bp, Artificial Sequence
  Synthetic
tcaacagatctgtcaaatcgcct

SEQ ID NO: 42 - DNA, 23 bp, Artificial Sequence
  Synthetic
ttcttctttctccaggctagaag

SEQ ID NO: 43 - DNA, 23 bp, Artificial Sequence
  Synthetic
gttcttctagcctggagaaagaa

SEQ ID NO: 44 - DNA, 23 bp, Artificial Sequence
  Synthetic
caaatcctgcattgttgcctgta

SEQ ID NO: 45 - DNA, 23 bp, Artificial Sequence
  Synthetic
ctgttaaagaggaagttagaaga

SEQ ID NO: 46 - DNA, 23 bp, Artificial Sequence
  Synthetic
aaaatttttatattacagaatat

SEQ ID NO: 47 - DNA, 23 bp, Artificial Sequence
  Synthetic
ttgtagactatcttttatattct

SEQ ID NO: 48 - DNA, 23 bp, Artificial Sequence
  Synthetic
ttttgcattttagatgaaagaga

SEQ ID NO: 49 - DNA, 23 bp, Artificial Sequence
  Synthetic
aacatcttctctttcatctaaaa

SEQ ID NO: 50 - DNA, 23 bp, Artificial Sequence
  Synthetic
ttttgaacatcttctctttcatc

SEQ ID NO: 51 - DNA, 23 bp, Artificial Sequence
  Synthetic
caaaaacccaaaatattttagct

SEQ ID NO: 52 - DNA, 23 bp, Artificial Sequence
  Synthetic
gcttgtgtttctaatttttcttt

SEQ ID NO: 53 - DNA, 23 bp, Artificial Sequence
  Synthetic
acttattgttattgaaattggct

SEQ ID NO: 54 - DNA, 23 bp, Artificial Sequence
  Synthetic
taccatgtattgctaaacaaagt

SEQ ID NO: 55 - DNA, 23 bp, Artificial Sequence
  Synthetic
gtatcaattcacaccagcaagtt

SEQ ID NO: 56 - DNA, 23 bp, Artificial Sequence
  Synthetic
ctcctctgtaaagtggcgattat

SEQ ID NO: 57 - DNA, 23 bp, Artificial Sequence
  Synthetic
tttaaaatgaagattttccacca

SEQ ID NO: 58 - DNA, 23 bp, Artificial Sequence
  Synthetic
aaatgaagattttccaccaatca

SEQ ID NO: 59 - DNA, 23 bp, Artificial Sequence
  Synthetic
ccaccaatcactttactctccta

SEQ ID NO: 60 - DNA, 23 bp, Artificial Sequence
  Synthetic
ccaccagttcttaggcaactgtt

SEQ ID NO: 61 - DNA, 23 bp, Artificial Sequence
  Synthetic
cattaatttatatccttgattat

SEQ ID NO: 62 - DNA, 23 bp, Artificial Sequence
  Synthetic
gttgttgttgttaaggtcaaagt

SEQ ID NO: 63 - DNA, 23 bp, Artificial Sequence
  Synthetic
aaattaccctagatcttaaagtt

SEQ ID NO: 64 - DNA, 24 bp, Artificial Sequence
  Synthetic
gcctctgattagggtgggggcgtg

SEQ ID NO: 65 - DNA, 24 bp, Artificial Sequence
  Synthetic
tcacaggctccaggaagggtttgg

SEQ ID NO: 66 - DNA, 24 bp, Artificial Sequence
  Synthetic
cccaggggggcctctttcggaagg

SEQ ID NO: 67 - DNA, 24 bp, Artificial Sequence
  Synthetic
ggaaggctctcttggtgatggaga

SEQ ID NO: 68 - DNA, 24 bp, Artificial Sequence
  Synthetic
aagctagtctagtgcaagctaaca

SEQ ID NO: 69 - DNA, 24 bp, Artificial Sequence
  Synthetic
ctggcctatgttattacctgtatg

SEQ ID NO: 70 - DNA, 24 bp, Artificial Sequence
  Synthetic
tggcctatgttattacctgtatgg

SEQ ID NO: 71 - DNA, 23 bp, Artificial Sequence
  Synthetic
ttccattctaatgggtggctgtt

SEQ ID NO: 72 - DNA, 20 bp, Artificial Sequence
  Synthetic
ctcctctgtaaagtggcgat

SEQ ID NO: 73 - DNA, 20 bp, Artificial Sequence
  Synthetic
ttccattctaatgggtggct

SEQ ID NO: 74 - DNA, 20 bp, Artificial Sequence
  Synthetic
gtatcaattcacaccagcaa

SEQ ID NO: 75 - DNA, 20 bp, Artificial Sequence
  Synthetic
taccatgtattgctaaacaa

SEQ ID NO: 76 - DNA, 20 bp, Artificial Sequence
  Synthetic
acttattgttattgaaattg

SEQ ID NO: 77 - DNA, 20 bp, Artificial Sequence
  Synthetic
gcttgtgtttctaatttttc

SEQ ID NO: 78 - DNA, 20 bp, Artificial Sequence
  Synthetic
caaaaacccaaaatatttta

SEQ ID NO: 79 - DNA, 20 bp, Artificial Sequence
  Synthetic
tttaaaatgaagattttcca

SEQ ID NO: 80 - DNA, 20 bp, Artificial Sequence
  Synthetic
aaatgaagattttccaccaa

SEQ ID NO: 81 - DNA, 20 bp, Artificial Sequence
  Synthetic
ccaccaatcactttactctc

SEQ ID NO: 82 - DNA, 20 bp, Artificial Sequence
  Synthetic
ccaccagttcttaggcaact

SEQ ID NO: 83 - DNA, 20 bp, Artificial Sequence
  Synthetic
cattaatttatatccttgat

SEQ ID NO: 84 - DNA, 20 bp, Artificial Sequence
  Synthetic
agttatagctctctttcaat

SEQ ID NO: 85 - DNA, 20 bp, Artificial Sequence
  Synthetic
atgtataacaattccaacat

SEQ ID NO: 86 - DNA, 20 bp, Artificial Sequence
  Synthetic
aaattaccctagatcttaaa

SEQ ID NO: 87 - DNA, 20 bp, Artificial Sequence
  Synthetic
gttgttgttgttaaggtcaa

SEQ ID NO: 88 - DNA, 20 bp, Artificial Sequence
  Synthetic
gcttgtgtttctaatttttc

SEQ ID NO: 89 - DNA, 20 bp, Artificial Sequence
  Synthetic
taatttttctttttcttctt

SEQ ID NO: 90 - DNA, 20 bp, Artificial Sequence
  Synthetic
gcaaaaaggaaaaaagaaga

SEQ ID NO: 91 - DNA, 20 bp, Artificial Sequence
  Synthetic
gggtttttgcaaaaaggaaa

SEQ ID NO: 92 - DNA, 20 bp, Artificial Sequence
  Synthetic
agctcctactcagactgtta

SEQ ID NO: 93 - DNA, 20 bp, Artificial Sequence
  Synthetic
tgcaaaaacccaaaatattt

SEQ ID NO: 94 - DNA, 20 bp, Artificial Sequence
  Synthetic
tgtcaccagagtaacagtct

SEQ ID NO: 95 - DNA, 20 bp, Artificial Sequence
  Synthetic
cttagtaaccacaggttgtg

SEQ ID NO: 96 - DNA, 20 bp, Artificial Sequence
  Synthetic
tagtttggagatggcagttt

SEQ ID NO: 97 - DNA, 20 bp, Artificial Sequence
  Synthetic
gagatggcagtttccttagt

SEQ ID NO: 98 - DNA, 20 bp, Artificial Sequence
  Synthetic
cttgatgttggaggtacctg

SEQ ID NO: 99 - DNA, 20 bp, Artificial Sequence
  Synthetic
atgttggaggtacctgctct

SEQ ID NO: 100 - DNA, 20 bp, Artificial Sequence
  Synthetic
taacttgatcaagcagagaa

SEQ ID NO: 101 - DNA, 20 bp, Artificial Sequence
  Synthetic
tctgcttgatcaagttataa

SEQ ID NO: 102 - DNA, 20 bp, Artificial Sequence
  Synthetic
taaaatcacagagggtgatg

SEQ ID NO: 103 - DNA, 20 bp, Artificial Sequence
  Synthetic
atatcctcaaggtcacccac

SEQ ID NO: 104 - DNA, 20 bp, Artificial Sequence
  Synthetic
atgatcatctcgttgatatc

SEQ ID NO: 105 - DNA, 20 bp, Artificial Sequence
  Synthetic
tcataccttctgcttgatga

SEQ ID NO: 106 - DNA, 20 bp, Artificial Sequence
  Synthetic
tcattttttctcataccttc

SEQ ID NO: 107 - DNA, 20 bp, Artificial Sequence
  Synthetic
tgccaacttttatcattttt

SEQ ID NO: 108 - DNA, 20 bp, Artificial Sequence
  Synthetic
aatcagaaagaagatcttat

SEQ ID NO: 109 - DNA, 20 bp, Artificial Sequence
  Synthetic
atttccctagggtccagctt

SEQ ID NO: 110 - DNA, 20 bp, Artificial Sequence
  Synthetic
gctcaaattgttactcttca

SEQ ID NO: 111 - DNA, 20 bp, Artificial Sequence
  Synthetic
agctcctactcagactgtta

SEQ ID NO: 112 - DNA, 20 bp, Artificial Sequence
  Synthetic
attctagtactatgcatctt

SEQ ID NO: 113 - DNA, 20 bp, Artificial Sequence
  Synthetic
acttaagttacttgtccagg

SEQ ID NO: 114 - DNA, 20 bp, Artificial Sequence
  Synthetic
ccaaggtcccagagttccta

SEQ ID NO: 115 - DNA, 20 bp, Artificial Sequence
  Synthetic
tttccctggcaaggtctgaa

SEQ ID NO: 116 - DNA, 20 bp, Artificial Sequence
  Synthetic
gctcattctcatgcctggac

SEQ ID NO: 117 - DNA, 20 bp, Artificial Sequence
  Synthetic
tttagcaatacatggtagaa

SEQ ID NO: 118 - DNA, 20 bp, Artificial Sequence
  Synthetic
agccaaactcttattcatga

SEQ ID NO: 119 - DNA, 20 bp, Artificial Sequence
  Synthetic
taacaatgtggatactttgt

SEQ ID NO: 120 - DNA, 4 bp, Artificial Sequence
  Synthetic
ttta

SEQ ID NO: 121 - DNA, 4 bp, Artificial Sequence
  Synthetic
tttg

SEQ ID NO: 122 - DNA, 4 bp, Artificial Sequence
  Synthetic
tttc

SEQ ID NO: 123 - DNA, 4 bp, Artificial Sequence
  Synthetic
tttt

SEQ ID NO: 124 - DNA, 9464 bp, Artificial Sequence
  Synthetic AsCpf1
gacggatcgggagatctcccgatcccctatggtgcactctcagtacaatctgctctgatgccgcatagttaagccagtatctgctccctgcttgtgtgttggaggtcgctgagtagtgcgcgagcaaaatttaagctacaacaaggcaaggcttgaccgacaattgcatgaagaatctgcttagggttaggcgttttgcgctgcttcgcgatgtacgggccagatatacgcgttgacattgattattgactagttattaatagtaatcaattacggggtcattagttcatagcccatatatggagttccgcgttacataacttacggtaaatggcccgcctggctgaccgcccaacgacccccgcccattgacgtcaataatgacgtatgttcccatagtaacgccaatagggactttccattgacgtcaatgggtggagtatttacggtaaactgcccacttggcagtacatcaagtgtatcatatgccaagtacgccccctattgacgtcaatgacggtaaatggcccgcctggcattatgcccagtacatgaccttatgggactttcctacttggcagtacatctacgtattagtcatcgctattaccatggtgatgcggttttggcagtacatcaatgggcgtggatagcggtttgactcacggggatttccaagtctccaccccattgacgtcaatgggagtttgttttggcaccaaaatcaacgggactttccaaaatgtcgtaacaactccgccccattgacgcaaatgggcggtaggcgtgtacggtgggaggtctatataagcagagctctctggctaactagagaacccactgcttactggcttatcgaaattaatacgactcactatagggagacccaagctggctagcgtttaaacttaagcttggtaccgccaccatgacacagttcgagggctttaccaacctgtatcaggtgagcaagacactgcggtttgagctgatcccacagggcaagaccctgaagcacatccaggagcagggcttcatcgaggaggacaaggcccgcaatgatcactacaaggagctgaagcccatcatcgatcggatctacaagacctatgccgaccagtgcctgcagctggtgcagctggattgggagaacctgagcgccgccatcgactcctatagaaaggagaaaaccgaggagacaaggaacgccctgatcgaggagcaggccacatatcgcaatgccatccacgactacttcatcggccggacagacaacctgaccgatgccatcaataagagacacgccgagatctacaagggcctgttcaaggccgagctgtttaatggcaaggtgctgaagcagctgggcaccgtgaccacaaccgagcacgagaacgccctgctgcggagcttcgacaagtttacaacctacttctccggcttttatgagaacaggaagaacgtgttcagcgccgaggatatcagcacagccatcccacaccgcatcgtgcaggacaacttccccaagtttaaggagaattgtcacatcttcacacgcctgatcaccgccgtgcccagcctgcgggagcactttgagaacgtgaagaaggccatcggcatcttcgtgagcacctccatcgaggaggtgttttccttccctttttataaccagctgctgacacagacccagatcgacctgtataaccagctgctgggaggaatctctcgggaggcaggcaccgagaagatcaagggcctgaacgaggtgctgaatctggccatccagaagaatgatgagacagcccacatcatcgcctccctgccacacagattcatccccctgtttaagcagatcctgtccgataggaacaccctgtctttcatcctggaggagtttaagagcgacgaggaagtgatccagtccttctgcaagtacaagacactgctgagaaacgagaacgtgctggagacagccgaggccctgtttaacgagctgaacagcatcgacctgacacacatcttcatcagccacaagaagctggagacaatcagcagcgccctgtgcgaccactgggatacactgaggaatgccctgtatgagcggagaatctccgagctgacaggcaagatcaccaagtctgccaaggagaaggtgcagcgcagcctgaagcacgaggatatcaacctgcaggagatcatctctgccgcaggcaaggagctgagcgaggccttcaagcagaaaaccagcgagatcctgtcccacgcacacgccgccctggatcagccactgcctacaaccctgaagaagcaggaggagaaggagatcctgaagtctcagctggacagcctgctgggcctgtaccacctgctggactggtttgccgtggatgagtccaacgaggtggaccccgagttctctgcccggctgaccggcatcaagctggagatggagccttctctgagcttctacaacaaggccagaaattatgccaccaagaagccctactccgtggagaagttcaagctgaactttcagatgcctacactggcctctggctgggacgtgaataaggagaagaacaatggcgccatcctgtttgtgaagaacggcctgtactatctgggcatcatgccaaagcagaagggcaggtataaggccctgagcttcgagcccacagagaaaaccagcgagggctttgataagatgtactatgactacttccctgatgccgccaagatgatcccaaagtgcagcacccagctgaaggccgtgacagcccactttcagacccacacaacccccatcctgctgtccaacaatttcatcgagcctctggagatcacaaaggagatctacgacctgaacaatcctgagaaggagccaaagaagtttcagacagcctacgccaagaaaaccggcgaccagaagggctacagagaggccctgtgcaagtggatcgacttcacaagggattttctgtccaagtataccaagacaacctctatcgatctgtctagcctgcggccatcctctcagtataaggacctgggcgagtactatgccgagctgaatcccctgctgtaccacatcagcttccagagaatcgccgagaaggagatcatggatgccgtggagacaggcaagctgtacctgttccagatctataacaaggactttgccaagggccaccacggcaagcctaatctgcacacactgtattggaccggcctgttttctccagagaacctggccaagacaagcatcaagctgaatggccaggccgagctgttctaccgccctaagtccaggatgaagaggatggcacaccggctgggagagaagatgctgaacaagaagctgaaggatcagaaaaccccaatccccgacaccctgtaccaggagctgtacgactatgtgaatcacagactgtcccacgacctgtctgatgaggccagggccctgctgcccaacgtgatcaccaaggaggtgtctcacgagatcatcaaggataggcgctttaccagcgacaagttctttttccacgtgcctatcacactgaactatcaggccgccaattccccatctaagttcaaccagagggtgaatgcctacctgaaggagcaccccgagacacctatcatcggcatcgatcggggcgagagaaacctgatctatatcacagtgatcgactccaccggcaagatcctggagcagcggagcctgaacaccatccagcagtttgattaccagaagaagctggacaacagggagaaggagagggtggcagcaaggcaggcctggtctgtggtgggcacaatcaaggatctgaagcagggctatctgagccaggtcatccacgagatcgtggacctgatgatccactaccaggccgtggtggtgctggagaacctgaatttcggctttaagagcaagaggaccggcatcgccgagaaggccgtgtaccagcagttcgagaagatgctgatcgataagctgaattgcctggtgctgaaggactatccagcagagaaagtgggaggcgtgctgaacccataccagctgacagaccagttcacctcctttgccaagatgggcacccagtctggcttcctgttttacgtgcctgccccatatacatctaagatcgatcccctgaccggcttcgtggaccccttcgtgtggaaaaccatcaagaatcacgagagccgcaagcacttcctggagggcttcgactttctgcactacgacgtgaaaaccggcgacttcatcctgcactttaagatgaacagaaatctgtccttccagaggggcctgcccggctttatgcctgcatgggatatcgtgttcgagaagaacgagacacagtttgacgccaagggcacccctttcatcgccggcaagagaatcgtgccagtgatcgagaatcacagattcaccggcagataccgggacctgtatcctgccaacgagctgatcgccctgctggaggagaagggcatcgtgttcagggatggctccaacatcctgccaaagctgctggagaatgacgattctcacgccatcgacaccatggtggccctgatccgcagcgtgctgcagatgcggaactccaatgccgccacaggcgaggactatatcaacagccccgtgcgcgatctgaatggcgtgtgcttcgactcccggtttcagaacccagagtggcccatggacgccgatgccaatggcgcctaccacatcgccctgaagggccagctgctgctgaatcacctgaaggagagcaaggatctgaagctgcagaacggcatctccaatcaggactggctggcctacatccaggagctgcgcaacaaaaggccggcggccacgaaaaaggccggccaggcaaaaaagaaaaagggatcctacccatacgatgttccagattacgcttatccctacgacgtgcctgattatgcatacccatatgatgtccccgactatgcctaagaattctgcagatatccagcacagtggcggccgctcgagtctagagggcccgtttaaacccgctgatcagcctcgactgtgccttctagttgccagccatctgttgtttgcccctcccccgtgccttccttgaccctggaaggtgccactcccactgtcctttcctaataaaatgaggaaattgcatcgcattgtctgagtaggtgtcattctattctggggggtggggtggggcaggacagcaagggggaggattgggaagacaatagcaggcatgctggggatgcggtgggctctatggcttctgaggcggaaagaaccagctggggctctagggggtatccccacgcgccctgtagcggcgcattaagcgcggcgggtgtggtggttacgcgcagcgtgaccgctacacttgccagcgccctagcgcccgctcctttcgctttcttcccttcctttctcgccacgttcgccggctttccccgtcaagctctaaatcgggggctccctttagggttccgatttagtgctttacggcacctcgaccccaaaaaacttgattagggtgatggttcacgtagtgggccatcgccctgatagacggtttttcgccctttgacgttggagtccacgttctttaatagtggactcttgttccaaactggaacaacactcaaccctatctcggtctattcttttgatttataagggattttgccgatttcggcctattggttaaaaaatgagctgatttaacaaaaatttaacgcgaattaattctgtggaatgtgtgtcagttagggtgtggaaagtccccaggctccccagcaggcagaagtatgcaaagcatgcatctcaattagtcagcaaccaggtgtggaaagtccccaggctccccagcaggcagaagtatgcaaagcatgcatctcaattagtcagcaaccatagtcccgcccctaactccgcccatcccgcccctaactccgcccagttccgcccattctccgccccatggctgactaattttttttatttatgcagaggccgaggccgcctctgcctctgagctattccagaagtagtgaggaggcttttttggaggcctaggcttttgcaaaaagctcccgggagcttgtatatccattttcggatctgatcaagagacaggatgaggatcgtttcgcatgattgaacaagatggattgcacgcaggttctccggccgcttgggtggagaggctattcggctatgactgggcacaacagacaatcggctgctctgatgccgccgtgttccggctgtcagcgcaggggcgcccggttctttttgtcaagaccgacctgtccggtgccctgaatgaactgcaggacgaggcagcgcggctatcgtggctggccacgacgggcgttccttgcgcagctgtgctcgacgttgtcactgaagcgggaagggactggctgctattgggcgaagtgccggggcaggatctcctgtcatctcaccttgctcctgccgagaaagtatccatcatggctgatgcaatgcggcggctgcatacgcttgatccggctacctgcccattcgaccaccaagcgaaacatcgcatcgagcgagcacgtactcggatggaagccggtcttgtcgatcaggatgatctggacgaagagcatcaggggctcgcgccagccgaactgttcgccaggctcaaggcgcgcatgcccgacggcgaggatctcgtcgtgacccatggcgatgcctgcttgccgaatatcatggtggaaaatggccgcttttctggattcatcgactgtggccggctgggtgtggcggaccgctatcaggacatagcgttggctacccgtgatattgctgaagagcttggcggcgaatgggctgaccgcttcctcgtgctttacggtatcgccgctcccgattcgcagcgcatcgccttctatcgccttcttgacgagttcttctgagcgggactctggggttcgaaatgaccgaccaagcgacgcccaacctgccatcacgagatttcgattccaccgccgccttctatgaaaggttgggcttcggaatcgttttccgggacgccggctggatgatcctccagcgcggggatctcatgctggagttcttcgcccaccccaacttgtttattgcagcttataatggttacaaataaagcaatagcatcacaaatttcacaaataaagcatttttttcactgcattctagttgtggtttgtccaaactcatcaatgtatcttatcatgtctgtataccgtcgacctctagctagagcttggcgtaatcatggtcatagctgtttcctgtgtgaaattgttatccgctcacaattccacacaacatacgagccggaagcataaagtgtaaagcctggggtgcctaatgagtgagctaactcacattaattgcgttgcgctcactgcccgctttccagtcgggaaacctgtcgtgccagctgcattaatgaatcggccaacgcgcggggagaggcggtttgcgtattgggcgctcttccgcttcctcgctcactgactcgctgcgctcggtcgttcggctgcggcgagcggtatcagctcactcaaaggcggtaatacggttatccacagaatcaggggataacgcaggaaagaacatgtgagcaaaaggccagcaaaaggccaggaaccgtaaaaaggccgcgttgctggcgtttttccataggctccgcccccctgacgagcatcacaaaaatcgacgctcaagtcagaggtggcgaaacccgacaggactataaagataccaggcgtttccccctggaagctccctcgtgcgctctcctgttccgaccctgccgcttaccggatacctgtccgcctttctcccttcgggaagcgtggcgctttctcatagctcacgctgtaggtatctcagttcggtgtaggtcgttcgctccaagctgggctgtgtgcacgaaccccccgttcagcccgaccgctgcgccttatccggtaactatcgtcttgagtccaacccggtaagacacgacttatcgccactggcagcagccactggtaacaggattagcagagcgaggtatgtaggcggtgctacagagttcttgaagtggtggcctaactacggctacactagaagaacagtatttggtatctgcgctctgctgaagccagttaccttcggaaaaagagttggtagctcttgatccggcaaacaaaccaccgctggtagcggtttttttgtttgcaagcagcagattacgcgcagaaaaaaaggatctcaagaagatcctttgatcttttctacggggtctgacgctcagtggaacgaaaactcacgttaagggattttggtcatgagattatcaaaaaggatcttcacctagatccttttaaattaaaaatgaagttttaaatcaatctaaagtatatatgagtaaacttggtctgacagttaccaatgcttaatcagtgaggcacctatctcagcgatctgtctatttcgttcatccatagttgcctgactccccgtcgtgtagataactacgatacgggagggcttaccatctggccccagtgctgcaatgataccgcgagacccacgctcaccggctccagatttatcagcaataaaccagccagccggaagggccgagcgcagaagtggtcctgcaactttatccgcctccatccagtctattaattgttgccgggaagctagagtaagtagttcgccagttaatagtttgcgcaacgttgttgccattgctacaggcatcgtggtgtcacgctcgtcgtttggtatggcttcattcagctccggttcccaacgatcaaggcgagttacatgatcccccatgttgtgcaaaaaagcggttagctccttcggtcctccgatcgttgtcagaagtaagttggccgcagtgttatcactcatggttatggcagcactgcataattctcttactgtcatgccatccgtaagatgcttttctgtgactggtgagtactcaaccaagtcattctgagaatagtgtatgcggcgaccgagttgctcttgcccggcgtcaatacgggataataccgcgccacatagcagaactttaaaagtgctcatcattggaaaacgttcttcggggcgaaaactctcaaggatcttaccgctgttgagatccagttcgatgtaacccactcgtgcacccaactgatcttcagcatcttttactttcaccagcgtttctgggtgagcaaaaacaggaaggcaaaatgccgcaaaaaagggaataagggcgacacggaaatgttgaatactcatactcttcctttttcaatattattgaagcatttatcagggttattgtctcatgagcggatacatatttgaatgtatttagaaaaataaacaaataggggttccgcgcacatttccccgaaaagtgccacctgacgtc

SEQ ID NO: 125 - DNA, 9227 bp, Artificial Sequence
  Synthetic LbCpf1
gacggatcgggagatctcccgatcccctatggtgcactctcagtacaatctgctctgatgccgcatagttaagccagtatctgctccctgcttgtgtgttggaggtcgctgagtagtgcgcgagcaaaatttaagctacaacaaggcaaggcttgaccgacaattgcatgaagaatctgcttagggttaggcgttttgcgctgcttcgcgatgtacgggccagatatacgcgttgacattgattattgactagttattaatagtaatcaattacggggtcattagttcatagcccatatatggagttccgcgttacataacttacggtaaatggcccgcctggctgaccgcccaacgacccccgcccattgacgtcaataatgacgtatgttcccatagtaacgccaatagggactttccattgacgtcaatgggtggagtatttacggtaaactgcccacttggcagtacatcaagtgtatcatatgccaagtacgccccctattgacgtcaatgacggtaaatggcccgcctggcattatgcccagtacatgaccttatgggactttcctacttggcagtacatctacgtattagtcatcgctattaccatggtgatgcggttttggcagtacatcaatgggcgtggatagcggtttgactcacggggatttccaagtctccaccccattgacgtcaatgggagtttgttttggcaccaaaatcaacgggactttccaaaatgtcgtaacaactccgccccattgacgcaaatgggcggtaggcgtgtacggtgggaggtctatataagcagagctctctggctaactagagaacccactgcttactggcttatcgaaattaatacgactcactatagggagacccaagctggctagcgtttaaacttaagcttggtaccgccaccatgagcaagctggagaagtttacaaactgctactccctgtctaagaccctgaggttcaaggccatccctgtgggcaagacccaggagaacatcgacaataagcggctgctggtggaggacgagaagagagccgaggattataagggcgtgaagaagctgctggatcgctactatctgtcttttatcaacgacgtgctgcacagcatcaagctgaagaatctgaacaattacatcagcctgttccggaagaaaaccagaaccgagaaggagaataaggagctggagaacctggagatcaatctgcggaaggagatcgccaaggccttcaagggcaacgagggctacaagtccctgtttaagaaggatatcatcgagacaatcctgccagagttcctggacgataaggacgagatcgccctggtgaacagcttcaatggctttaccacagccttcaccggcttctttgataacagagagaatatgttttccgaggaggccaagagcacatccatcgccttcaggtgtatcaacgagaatctgacccgctacatctctaatatggacatcttcgagaaggtggacgccatctttgataagcacgaggtgcaggagatcaaggagaagatcctgaacagcgactatgatgtggaggatttctttgagggcgagttctttaactttgtgctgacacaggagggcatcgacgtgtataacgccatcatcggcggcttcgtgaccgagagcggcgagaagatcaagggcctgaacgagtacatcaacctgtataatcagaaaaccaagcagaagctgcctaagtttaagccactgtataagcaggtgctgagcgatcgggagtctctgagcttctacggcgagggctatacatccgatgaggaggtgctggaggtgtttagaaacaccctgaacaagaacagcgagatcttcagctccatcaagaagctggagaagctgttcaagaattttgacgagtactctagcgccggcatctttgtgaagaacggccccgccatcagcacaatctccaaggatatcttcggcgagtggaacgtgatccgggacaagtggaatgccgagtatgacgatatccacctgaagaagaaggccgtggtgaccgagaagtacgaggacgatcggagaaagtccttcaagaagatcggctccttttctctggagcagctgcaggagtacgccgacgccgatctgtctgtggtggagaagctgaaggagatcatcatccagaaggtggatgagatctacaaggtgtatggctcctctgagaagctgttcgacgccgattttgtgctggagaagagcctgaagaagaacgacgccgtggtggccatcatgaaggacctgctggattctgtgaagagcttcgagaattacatcaaggccttctttggcgagggcaaggagacaaacagggacgagtccttctatggcgattttgtgctggcctacgacatcctgctgaaggtggaccacatctacgatgccatccgcaattatgtgacccagaagccctactctaaggataagttcaagctgtattttcagaaccctcagttcatgggcggctgggacaaggataaggagacagactatcgggccaccatcctgagatacggctccaagtactatctggccatcatggataagaagtacgccaagtgcctgcagaagatcgacaaggacgatgtgaacggcaattacgagaagatcaactataagctgctgcccggccctaataagatgctgccaaaggtgttcttttctaagaagtggatggcctactataaccccagcgaggacatccagaagatctacaagaatggcacattcaagaagggcgatatgtttaacctgaatgactgtcacaagctgatcgacttctttaaggatagcatctcccggtatccaaagtggtccaatgcctacgatttcaacttttctgagacagagaagtataaggacatcgccggcttttacagagaggtggaggagcagggctataaggtgagcttcgagtctgccagcaagaaggaggtggataagctggtggaggagggcaagctgtatatgttccagatctataacaaggacttttccgataagtctcacggcacacccaatctgcacaccatgtacttcaagctgctgtttgacgagaacaatcacggacagatcaggctgagcggaggagcagagctgttcatgaggcgcgcctccctgaagaaggaggagctggtggtgcacccagccaactcccctatcgccaacaagaatccagataatcccaagaaaaccacaaccctgtcctacgacgtgtataaggataagaggttttctgaggaccagtacgagctgcacatcccaatcgccatcaataagtgccccaagaacatcttcaagatcaatacagaggtgcgcgtgctgctgaagcacgacgataacccctatgtgatcggcatcgataggggcgagcgcaatctgctgtatatcgtggtggtggacggcaagggcaacatcgtggagcagtattccctgaacgagatcatcaacaacttcaacggcatcaggatcaagacagattaccactctctgctggacaagaaggagaaggagaggttcgaggcccgccagaactggacctccatcgagaatatcaaggagctgaaggccggctatatctctcaggtggtgcacaagatctgcgagctggtggagaagtacgatgccgtgatcgccctggaggacctgaactctggctttaagaatagccgcgtgaaggtggagaagcaggtgtatcagaagttcgagaagatgctgatcgataagctgaactacatggtggacaagaagtctaatccttgtgcaacaggcggcgccctgaagggctatcagatcaccaataagttcgagagctttaagtccatgtctacccagaacggcttcatcttttacatccctgcctggctgacatccaagatcgatccatctaccggctttgtgaacctgctgaaaaccaagtataccagcatcgccgattccaagaagttcatcagctcctttgacaggatcatgtacgtgcccgaggaggatctgttcgagtttgccctggactataagaacttctctcgcacagacgccgattacatcaagaagtggaagctgtactcctacggcaaccggatcagaatcttccggaatcctaagaagaacaacgtgttcgactgggaggaggtgtgcctgaccagcgcctataaggagctgttcaacaagtacggcatcaattatcagcagggcgatatcagagccctgctgtgcgagcagtccgacaaggccttctactctagctttatggccctgatgagcctgatgctgcagatgcggaacagcatcacaggccgcaccgacgtggattttctgatcagccctgtgaagaactccgacggcatcttctacgatagccggaactatgaggcccaggagaatgccatcctgccaaagaacgccgacgccaatggcgcctataacatcgccagaaaggtgctgtgggccatcggccagttcaagaaggccgaggacgagaagctggataaggtgaagatcgccatctctaacaaggagtggctggagtacgcccagaccagcgtgaagcacaaaaggccggcggccacgaaaaaggccggccaggcaaaaaagaaaaagggatcctacccatacgatgttccagattacgcttatccctacgacgtgcctgattatgcatacccatatgatgtccccgactatgcctaagaattctgcagatatccagcacagtggcggccgctcgagtctagagggcccgtttaaacccgctgatcagcctcgactgtgccttctagttgccagccatctgttgtttgcccctcccccgtgccttccttgaccctggaaggtgccactcccactgtcctttcctaataaaatgaggaaattgcatcgcattgtctgagtaggtgtcattctattctggggggtggggtggggcaggacagcaagggggaggattgggaagacaatagcaggcatgctggggatgcggtgggctctatggcttctgaggcggaaagaaccagctggggctctagggggtatccccacgcgccctgtagcggcgcattaagcgcggcgggtgtggtggttacgcgcagcgtgaccgctacacttgccagcgccctagcgcccgctcctttcgctttcttcccttcctttctcgccacgttcgccggctttccccgtcaagctctaaatcgggggctccctttagggttccgatttagtgctttacggcacctcgaccccaaaaaacttgattagggtgatggttcacgtagtgggccatcgccctgatagacggtttttcgccctttgacgttggagtccacgttctttaatagtggactcttgttccaaactggaacaacactcaaccctatctcggtctattcttttgatttataagggattttgccgatttcggcctattggttaaaaaatgagctgatttaacaaaaatttaacgcgaattaattctgtggaatgtgtgtcagttagggtgtggaaagtccccaggctccccagcaggcagaagtatgcaaagcatgcatctcaattagtcagcaaccaggtgtggaaagtccccaggctccccagcaggcagaagtatgcaaagcatgcatctcaattagtcagcaaccatagtcccgcccctaactccgcccatcccgcccctaactccgcccagttccgcccattctccgccccatggctgactaattttttttatttatgcagaggccgaggccgcctctgcctctgagctattccagaagtagtgaggaggcttttttggaggcctaggcttttgcaaaaagctcccgggagcttgtatatccattttcggatctgatcaagagacaggatgaggatcgtttcgcatgattgaacaagatggattgcacgcaggttctccggccgcttgggtggagaggctattcggctatgactgggcacaacagacaatcggctgctctgatgccgccgtgttccggctgtcagcgcaggggcgcccggttctttttgtcaagaccgacctgtccggtgccctgaatgaactgcaggacgaggcagcgcggctatcgtggctggccacgacgggcgttccttgcgcagctgtgctcgacgttgtcactgaagcgggaagggactggctgctattgggcgaagtgccggggcaggatctcctgtcatctcaccttgctcctgccgagaaagtatccatcatggctgatgcaatgcggcggctgcatacgcttgatccggctacctgcccattcgaccaccaagcgaaacatcgcatcgagcgagcacgtactcggatggaagccggtcttgtcgatcaggatgatctggacgaagagcatcaggggctcgcgccagccgaactgttcgccaggctcaaggcgcgcatgcccgacggcgaggatctcgtcgtgacccatggcgatgcctgcttgccgaatatcatggtggaaaatggccgcttttctggattcatcgactgtggccggctgggtgtggcggaccgctatcaggacatagcgttggctacccgtgatattgctgaagagcttggcggcgaatgggctgaccgcttcctcgtgctttacggtatcgccgctcccgattcgcagcgcatcgccttctatcgccttcttgacgagttcttctgagcgggactctggggttcgaaatgaccgaccaagcgacgcccaacctgccatcacgagatttcgattccaccgccgccttctatgaaaggttgggcttcggaatcgttttccgggacgccggctggatgatcctccagcgcggggatctcatgctggagttcttcgcccaccccaacttgtttattgcagcttataatggttacaaataaagcaatagcatcacaaatttcacaaataaagcatttttttcactgcattctagttgtggtttgtccaaactcatcaatgtatcttatcatgtctgtataccgtcgacctctagctagagcttggcgtaatcatggtcatagctgtttcctgtgtgaaattgttatccgctcacaattccacacaacatacgagccggaagcataaagtgtaaagcctggggtgcctaatgagtgagctaactcacattaattgcgttgcgctcactgcccgctttccagtcgggaaacctgtcgtgccagctgcattaatgaatcggccaacgcgcggggagaggcggtttgcgtattgggcgctcttccgcttcctcgctcactgactcgctgcgctcggtcgttcggctgcggcgagcggtatcagctcactcaaaggcggtaatacggttatccacagaatcaggggataacgcaggaaagaacatgtgagcaaaaggccagcaaaaggccaggaaccgtaaaaaggccgcgttgctggcgtttttccataggctccgcccccctgacgagcatcacaaaaatcgacgctcaagtcagaggtggcgaaacccgacaggactataaagataccaggcgtttccccctggaagctccctcgtgcgctctcctgttccgaccctgccgcttaccggatacctgtccgcctttctcccttcgggaagcgtggcgctttctcatagctcacgctgtaggtatctcagttcggtgtaggtcgttcgctccaagctgggctgtgtgcacgaaccccccgttcagcccgaccgctgcgccttatccggtaactatcgtcttgagtccaacccggtaagacacgacttatcgccactggcagcagccactggtaacaggattagcagagcgaggtatgtaggcggtgctacagagttcttgaagtggtggcctaactacggctacactagaagaacagtatttggtatctgcgctctgctgaagccagttaccttcggaaaaagagttggtagctcttgatccggcaaacaaaccaccgctggtagcggtttttttgtttgcaagcagcagattacgcgcagaaaaaaaggatctcaagaagatcctttgatcttttctacggggtctgacgctcagtggaacgaaaactcacgttaagggattttggtcatgagattatcaaaaaggatcttcacctagatccttttaaattaaaaatgaagttttaaatcaatctaaagtatatatgagtaaacttggtctgacagttaccaatgcttaatcagtgaggcacctatctcagcgatctgtctatttcgttcatccatagttgcctgactccccgtcgtgtagataactacgatacgggagggcttaccatctggccccagtgctgcaatgataccgcgagacccacgctcaccggctccagatttatcagcaataaaccagccagccggaagggccgagcgcagaagtggtcctgcaactttatccgcctccatccagtctattaattgttgccgggaagctagagtaagtagttcgccagttaatagtttgcgcaacgttgttgccattgctacaggcatcgtggtgtcacgctcgtcgtttggtatggcttcattcagctccggttcccaacgatcaaggcgagttacatgatcccccatgttgtgcaaaaaagcggttagctccttcggtcctccgatcgttgtcagaagtaagttggccgcagtgttatcactcatggttatggcagcactgcataattctcttactgtcatgccatccgtaagatgcttttctgtgactggtgagtactcaaccaagtcattctgagaatagtgtatgcggcgaccgagttgctcttgcccggcgtcaatacgggataataccgcgccacatagcagaactttaaaagtgctcatcattggaaaacgttcttcggggcgaaaactctcaaggatcttaccgctgttgagatccagttcgatgtaacccactcgtgcacccaactgatcttcagcatcttttactttcaccagcgtttctgggtgagcaaaaacaggaaggcaaaatgccgcaaaaaagggaataagggcgacacggaaatgttgaatactcatactcttcctttttcaatattattgaagcatttatcagggttattgtctcatgagcggatacatatttgaatgtatttagaaaaataaacaaataggggttccgcgcacatttccccgaaaagtgccacctgacgtc